European Patent Specification EP 3 456 345 B1, published March 26, 2025. Title: Sheep Nematode Vaccine. Applicant: Moredun research Institute Matthews, Jacqueline Nisbet, Alasdair J Knox, David J. The sequence listing filed with the application follows.

SEQUENCE LISTING (8 sequences)

SEQ ID NO: 1 - protein, 162 aa, Teladorsagia circumcincta
MFCRVTVAVLLLAVSAHAGFFDDVSGLASDVGDFFTKQFNNVKDLFANNQSELEKNIQRVKDLLMAIKEKAKMLEPMANDAQKKTISEVNNYMQQVDAFGAQVKRDGEAKFEQNKAKWQDMLNNIFEKGGLENVMKLMNLKSATQCTVMAALIAPVILAFTR

SEQ ID NO: 2 - protein, 115 aa, Teladorsagia circumcincta
MPVFSFHTNVSADKVTPDLLKQISSVVARILHKPESYVCVHVVPDQQMIFDGTDGPCGVGVLKSIGGVGGSKNNEHAKALFALIKDHLGIAGNRMYIEFIDIGAADIAFNSRTFA

SEQ ID NO: 3 - protein, 236 aa, Teladorsagia circumcincta
MFTPIGIAVLYLALVTPHAKAGFCCPADLDQTDEARKILLNFHNEVRRDVSSASPLLNLTGAVLMRNVLGPAKNMYKMDWDCNLEKKALEMISPCTVPLPIDTSIPQNLAQWLLYRKMEETEVLEKAPWSWVIASLRNLKNDTEADLYNWKIRTISNILNWRNTKVGCAHKVCQFPTGTNMVISCAYGGDKLENNEVVWQKGPTCECNAYPDSYCCNNLCDTKAAAALREEPCKSN

SEQ ID NO: 4 - protein, 305 aa, Teladorsagia circumcincta
MRLLNSMGMQEPPNVDSIDLSPSTIEEMLESLGENDKLEQDQEEKTFIMAVDPSDGIDPDMLVARFPVSITTMVRKVSRAYLHVYLHVSEPLPEPEIVTVVVRERLLNGDVGDIVATNPVEIQRSGKAVLPLRASDVERWWKSEPILGLYVVAMLNGENIAVHPQQDHHARHTMFMSVILASDAKSRGKRSPSVCMPEDQEPGCCLYDLIVDFQQIGWKFIIAPHKYNAYMCRGDCSVNHTHVTRSGHTKVAKTGIITRQDATGNQGMCCHPAEYDAVRMIYMNGDNQVTMARVPGMIARKCTCS

SEQ ID NO: 5 - protein, 364 aa, Teladorsagia circumcincta
MSLLFLLLIPHLFAATVKQQYSGGVKPLTELRTDLIDKKTKGSIEFARLGQHISPKDFGAWNHFTSFIERHDKVYRNESEALKRFGIFKRNLEIIRSAQENDKGTAIYGINQFADLSPEEFKKTHLPHTWKQPDHPNRIVDLAAEGVDPKEPLPESFDWREHGAVTKVKTEGHCAACWAFSVTGNIEGQWFLAKKKLVSLSAQQLLDCDVVDEGCNGGFPLDAYKEIVRMGGLEPEDKYPYEAKAEQCRLVPSDIAVYINGSVELPHDEEKMRAWLVKKGPISIGITVDDIQFYKGGVSRPTTCRLSSMIHGALLVGYGVEKNIPYWIIKNSWGPNWGEDGYYRMVRGENACRINRFPTSAVVL

SEQ ID NO: 6 - protein, 339 aa, Teladorsagia circumcincta
MLLYILSLVLLIDALPPGYPDGKEHGSRPTIRSLPDGSTEYKLLIVTDMDKDSKAGEWTWRAVTREGRLTLSPDMAHVSIAWDENSERNLTSSMNIKGRAMELSDLSVFHNRILTPDDRTGLISEIKNNKMIPWVFLNSGPGNTTSPFKCEWMTIKDDVLYVGGHGNEFRNKQGEIVHRNNLWIKTVTPEGEVTNVDWTDVFNNLRNAVGISEPGYLTHEAVQWSEKQGHWYFLPRKESKTVYVEEDDEKKGTDLLIIGNPDLDQFETKRIGVLRPERGYSAFDFIPGTDDKIIVALKSKEVTDEPTETYVTVFTIDGEILLDDQKLDGNYKFEGLYFI

SEQ ID NO: 7 - protein, 498 aa, Teladorsagia circumcincta
MRLAVLLLVLVVSAQAGLLDKVKDFFKGGNFGEKTKTATLSKFKKLFEKTGILSLGNKLAEMRSKVMKKLELSKAKKAEVDRKLKEVEERMDNTVENLKDTIFEINAVKNVGESLFQSDILLTKRQVEEVMDGVEGGRPKRQAFKDQNYPNTTWQQGVFYRFDDSADYYTRKVFEMGTKQWEEATCIDFKEDKEKKAENSIILIKEDGCWSYVGQVGGEQPLSLGDGCEQVGIATHELGHALGLFHTMSRYDRDDFITVVLENVVEGFVDQYIKETPQTTTNYGFTYDYGSIMHYGASSASHNNKPTMVANDTRYQESMGSQIISFIDKSMINDHYNCKADCPKATSAKCQNGGFPHPRKCSECICPSGYGGALCDQRPTGCGQTLKAKESKQFLIDKLGFPSGVRDEFTFCNHWIEAPEGKKIELKINSISHGYAHDGCILGGVEIKTSEDQTRTGFRFCSPNDRNTVLVSASNRVPIITFNRSGQQQIILEYKVVS

SEQ ID NO: 8 - protein, 160 aa, Teladorsagia circumcincta
MLRSILLILVSASVYVSVQGQGNGDMKKVELYMGYAKKDMEKVREFLKLKDERLTKLLSDLFRYLDKTTFEWMKDEATLEQFIQTRGKFSSALVHPDVQKRYKDNRKLWAFRYARLMNCIGGSDMGRATAYLPGVSVQEKEETLRYSLKLERTCAYTYFR